European Patent Application EP 4 357 363 A1, published April 24, 2024. Title: ANTI-TM4SF4 HUMANIZED ANTIBODIES AND USE THEREOF. Applicant: KOREA ATOMIC ENERGY RESEARCH INSTITUTE INDUSTRY ACADEMY COOPERATION FOUNDATION OF SEJONG UNIVERSITY. The sequence listing filed with the application follows.

SEQUENCE LISTING (80 sequences)

SEQ ID NO: 1 - protein, 30 aa, Artificial Sequence
  Hz2B7-1.0~4.0 FR1
EITLKESGPTLVKPTQTLTLTCTFSGFSLS

SEQ ID NO: 2 - protein, 14 aa, Artificial Sequence
  Hz2B7-1.0,3.0,4.0 FR2
WIRQPPGKALEWLA

SEQ ID NO: 3 - protein, 14 aa, Artificial Sequence
  Hz2B7-2.0 FR2
WIRQPPGKVLEWLA

SEQ ID NO: 4 - protein, 32 aa, Artificial Sequence
  Hz2B7-1.0~4.0 FR3
RLTITKDTSKNQVVLTMTNMDPVDTATYYCAR

SEQ ID NO: 5 - protein, 11 aa, Artificial Sequence
  Hz2B7-1.0~4.0 FR4
WGQGTLVTVSS

SEQ ID NO: 6 - protein, 23 aa, Artificial Sequence
  Hz2B7-0.1~0.3 FR1
DIVMTQSPDSLAVSLGERATINC

SEQ ID NO: 7 - protein, 15 aa, Artificial Sequence
  Hz2B7-0.1~0.3 FR2
WYQQKPGQPPKLLIY

SEQ ID NO: 8 - protein, 32 aa, Artificial Sequence
  Hz2B7-0.1~0.3 FR3
GVPDRFSGSGSGTDFTLTISLMQAEDVAVYYC

SEQ ID NO: 9 - protein, 10 aa, Artificial Sequence
  Hz2B7-0.1~0.3 FR4
FGQGTKVEIK

SEQ ID NO: 10 - protein, 7 aa, Artificial Sequence
  Hz2B7-1.0~4.0 CDR1
TYGIGVS

SEQ ID NO: 11 - protein, 16 aa, Artificial Sequence
  Hz2B7-1.0,2.0 CDR2
HIWWNDNKYYNTALKS

SEQ ID NO: 12 - protein, 16 aa, Artificial Sequence
  Hz2B7-3.0 CDR2
HIWSNDNKYYNTALKS

SEQ ID NO: 13 - protein, 16 aa, Artificial Sequence
  Hz2B7-4.0 CDR2
HIWYNDNKYYNTALKS

SEQ ID NO: 14 - protein, 10 aa, Artificial Sequence
  Hz2B7-1.0~4.0 CDR3
KEGSSAPFAY

SEQ ID NO: 15 - protein, 17 aa, Artificial Sequence
  Hz2B7-0.1 CDR1
KSSQSLLNSSNQKNYLA

SEQ ID NO: 16 - protein, 17 aa, Artificial Sequence
  Hz2B7-0.2 CDR1
KSSQSLLFSSNQKNYLA

SEQ ID NO: 17 - protein, 17 aa, Artificial Sequence
  Hz2B7-0.3 CDR1
KSSQSLLVSSNQKNYLA

SEQ ID NO: 18 - protein, 7 aa, Artificial Sequence
  Hz2B7-0.1~0.3 CDR2
FASTRES

SEQ ID NO: 19 - protein, 9 aa, Artificial Sequence
  Hz2B7-0.1~0.3 CDR3
QQHYRTPPT

SEQ ID NO: 20 - protein, 120 aa, Artificial Sequence
  Hz2B7-1.0
EITLKESGPTLVKPTQTLTLTCTFSGFSLSTYGIGVSWIRQPPGKALEWLAHIWWNDNKYYNTALKSRLTITKDTSKNQVVLTMTNMDPVDTATYYCARKEGSSAPFAYWGQGTLVTVSS

SEQ ID NO: 21 - protein, 120 aa, Artificial Sequence
  Hz2B7-2.0
EITLKESGPTLVKPTQTLTLTCTFSGFSLSTYGIGVSWIRQPPGKVLEWLAHIWWNDNKYYNTALKSRLTITKDTSKNQVVLTMTNMDPVDTATYYCARKEGSSAPFAYWGQGTLVTVSS

SEQ ID NO: 22 - protein, 120 aa, Artificial Sequence
  Hz2B7-3.0
EITLKESGPTLVKPTQTLTLTCTFSGFSLSTYGIGVSWIRQPPGKALEWLAHIWSNDNKYYNTALKSRLTITKDTSKNQVVLTMTNMDPVDTATYYCARKEGSSAPFAYWGQGTLVTVSS

SEQ ID NO: 23 - protein, 120 aa, Artificial Sequence
  Hz2B7-4.0
EITLKESGPTLVKPTQTLTLTCTFSGFSLSTYGIGVSWIRQPPGKALEWLAHIWYNDNKYYNTALKSRLTITKDTSKNQVVLTMTNMDPVDTATYYCARKEGSSAPFAYWGQGTLVTVSS

SEQ ID NO: 24 - protein, 113 aa, Artificial Sequence
  Hz2B7-0.1
DIVMTQSPDSLAVSLGERATINCKSSQSLLNSSNQKNYLAWYQQKPGQPPKLLIYFASTRESGVPDRFSGSGSGTDFTLTISLMQAEDVAVYYCQQHYRTPPTFGQGTKVEIK

SEQ ID NO: 25 - protein, 113 aa, Artificial Sequence
  Hz2B7-0.2
DIVMTQSPDSLAVSLGERATINCKSSQSLLFSSNQKNYLAWYQQKPGQPPKLLIYFASTRESGVPDRFSGSGSGTDFTLTISLMQAEDVAVYYCQQHYRTPPTFGQGTKVEIK

SEQ ID NO: 26 - protein, 113 aa, Artificial Sequence
  Hz2B7-0.3
DIVMTQSPDSLAVSLGERATINCKSSQSLLVSSNQKNYLAWYQQKPGQPPKLLIYFASTRESGVPDRFSGSGSGTDFTLTISLMQAEDVAVYYCQQHYRTPPTFGQGTKVEIK

SEQ ID NO: 27 - protein, 330 aa, Artificial Sequence [sequence omitted]

SEQ ID NO: 28 - protein, 107 aa, Artificial Sequence [sequence omitted]

SEQ ID NO: 29 - DNA, 90 bp, Artificial Sequence
  Hz2B7-1.0~4.0 FR1
gagatcaccctgaaggagagcggccccaccctggtgaagcccacccagaccctgaccctgacctgcaccttcagcggcttcagcctgagc

SEQ ID NO: 30 - DNA, 42 bp, Artificial Sequence
  Hz2B7-1.0,3.0,4.0 FR2
tggatcaggcagccccccggcaaggccctggagtggctggcc

SEQ ID NO: 31 - DNA, 42 bp, Artificial Sequence
  Hz2B7-2.0 FR2
tggatcaggcagccccccggcaaggtcctggagtggctggcc

SEQ ID NO: 32 - DNA, 96 bp, Artificial Sequence
  Hz2B7-1.0~4.0 FR3
aggctgaccatcaccaaggacaccagcaagaaccaggtggtgctgaccatgaccaacatggaccccgtggacaccgccacctactactgcgccagg

SEQ ID NO: 33 - DNA, 33 bp, Artificial Sequence
  Hz2B7-1.0~4.0 FR4
tggggccagggcaccctggtgaccgtgagcagc

SEQ ID NO: 34 - DNA, 69 bp, Artificial Sequence
  Hz2B7-0.1~0.3 FR1
gacatcgtgatgacccagagccccgacagcctggccgtgagcctgggcgagagggccaccatcaactgc

SEQ ID NO: 35 - DNA, 45 bp, Artificial Sequence
  Hz2B7-0.1~0.3 FR2
tggtaccagcagaagcccggccagccccccaagctgctgatctac

SEQ ID NO: 36 - DNA, 96 bp, Artificial Sequence
  Hz2B7-0.1~0.3 FR3
ggcgtgcccgacaggttcagcggcagcggcagcggcaccgacttcaccctgaccatcagcagcctgcaggccgaggacgtggccgtgtactactgc

SEQ ID NO: 37 - DNA, 30 bp, Artificial Sequence
  Hz2B7-0.1~0.3 FR4
ttcggccagggcaccaaggtggagatcaag

SEQ ID NO: 38 - DNA, 21 bp, Artificial Sequence
  Hz2B7-1.0~4.0 CDR1
acttatggtataggagtaagc

SEQ ID NO: 39 - DNA, 48 bp, Artificial Sequence
  Hz2B7-1.0,2.0 CDR2
cacatttggtggaatgataataagtactataacacagccctgaagagc

SEQ ID NO: 40 - DNA, 48 bp, Artificial Sequence
  Hz2B7-3.0 CDR2
cacatttggtcgaatgataataagtactataacacagccctgaagagc

SEQ ID NO: 41 - DNA, 48 bp, Artificial Sequence
  Hz2B7-4.0 CDR2
cacatttggtataatgataataagtactataacacagccctgaagagc

SEQ ID NO: 42 - DNA, 30 bp, Artificial Sequence
  Hz2B7-1.0~4.0 CDR3
aaggagggcagctcggccccctttgcttac

SEQ ID NO: 43 - DNA, 51 bp, Artificial Sequence
  Hz2B7-0.1 CDR1
aagtccagtcagagccttttaaatagtagcaatcaaaagaactatttggcc

SEQ ID NO: 44 - DNA, 51 bp, Artificial Sequence
  Hz2B7-0.2 CDR1
aagtccagtcagagccttttattcagtagcaatcaaaagaactatttggcc

SEQ ID NO: 45 - DNA, 51 bp, Artificial Sequence
  Hz2B7-0.3 CDR1
aagtccagtcagagccttttagtaagtagcaatcaaaagaactatttggcc

SEQ ID NO: 46 - DNA, 21 bp, Artificial Sequence
  Hz2B7-0.1~0.3 CDR2
tttgcatccactagggaatct

SEQ ID NO: 47 - DNA, 27 bp, Artificial Sequence
  Hz2B7-0.1~0.3 CDR3
cagcaacattatagaactcctccgacg

SEQ ID NO: 48 - DNA, 360 bp, Artificial Sequence
  Hz2B7-1.0
gagatcaccctgaaggagagcggccccaccctggtgaagcccacccagaccctgaccctgacctgcaccttcagcggcttcagcctgagcacttatggtataggagtaagctggatcaggcagccccccggcaaggccctggagtggctggcccacatttggtggaatgataataagtactataacacagccctgaagagcaggctgaccatcaccaaggacaccagcaagaaccaggtggtgctgaccatgaccaacatggaccccgtggacaccgccacctactactgcgccaggaaggagggcagctcggccccctttgcttactggggccagggcaccctggtgaccgtgagcagc

SEQ ID NO: 49 - DNA, 360 bp, Artificial Sequence
  Hz2B7-2.0
gagatcaccctgaaggagagcggccccaccctggtgaagcccacccagaccctgaccctgacctgcaccttcagcggcttcagcctgagcacttatggtataggagtaagctggatcaggcagccccccggcaaggtcctggagtggctggcccacatttggtggaatgataataagtactataacacagccctgaagagcaggctgaccatcaccaaggacaccagcaagaaccaggtggtgctgaccatgaccaacatggaccccgtggacaccgccacctactactgcgccaggaaggagggcagctcggccccctttgcttactggggccagggcaccctggtgaccgtgagcagc

SEQ ID NO: 50 - DNA, 360 bp, Artificial Sequence
  Hz2B7-3.0
gagatcaccctgaaggagagcggccccaccctggtgaagcccacccagaccctgaccctgacctgcaccttcagcggcttcagcctgagcacttatggtataggagtaagctggatcaggcagccccccggcaaggccctggagtggctggcccacatttggtcgaatgataataagtactataacacagccctgaagagcaggctgaccatcaccaaggacaccagcaagaaccaggtggtgctgaccatgaccaacatggaccccgtggacaccgccacctactactgcgccaggaaggagggcagctcggccccctttgcttactggggccagggcaccctggtgaccgtgagcagc

SEQ ID NO: 51 - DNA, 360 bp, Artificial Sequence
  Hz2B7-4.0
gagatcaccctgaaggagagcggccccaccctggtgaagcccacccagaccctgaccctgacctgcaccttcagcggcttcagcctgagcacttatggtataggagtaagctggatcaggcagccccccggcaaggccctggagtggctggcccacatttggtataatgataataagtactataacacagccctgaagagcaggctgaccatcaccaaggacaccagcaagaaccaggtggtgctgaccatgaccaacatggaccccgtggacaccgccacctactactgcgccaggaaggagggcagctcggccccctttgcttactggggccagggcaccctggtgaccgtgagcagc

SEQ ID NO: 52 - DNA, 339 bp, Artificial Sequence
  Hz2B7-0.1
gacatcgtgatgacccagagccccgacagcctggccgtgagcctgggcgagagggccaccatcaactgcaagtccagtcagagccttttaaatagtagcaatcaaaagaactatttggcctggtaccagcagaagcccggccagccccccaagctgctgatctactttgcatccactagggaatctggcgtgcccgacaggttcagcggcagcggcagcggcaccgacttcaccctgaccatcagcagcctgcaggccgaggacgtggccgtgtactactgccagcaacattatagaactcctccgacgttcggccagggcaccaaggtggagatcaag

SEQ ID NO: 53 - DNA, 339 bp, Artificial Sequence
  Hz2B7-0.2
gacatcgtgatgacccagagccccgacagcctggccgtgagcctgggcgagagggccaccatcaactgcaagtccagtcagagccttttattcagtagcaatcaaaagaactatttggcctggtaccagcagaagcccggccagccccccaagctgctgatctactttgcatccactagggaatctggcgtgcccgacaggttcagcggcagcggcagcggcaccgacttcaccctgaccatcagcagcctgcaggccgaggacgtggccgtgtactactgccagcaacattatagaactcctccgacgttcggccagggcaccaaggtggagatcaag

SEQ ID NO: 54 - DNA, 339 bp, Artificial Sequence
  Hz2B7-0.3
gacatcgtgatgacccagagccccgacagcctggccgtgagcctgggcgagagggccaccatcaactgcaagtccagtcagagccttttagtaagtagcaatcaaaagaactatttggcctggtaccagcagaagcccggccagccccccaagctgctgatctactttgcatccactagggaatctggcgtgcccgacaggttcagcggcagcggcagcggcaccgacttcaccctgaccatcagcagcctgcaggccgaggacgtggccgtgtactactgccagcaacattatagaactcctccgacgttcggccagggcaccaaggtggagatcaag

SEQ ID NO: 55 - DNA, 990 bp, Artificial Sequence
  Heavy chain constant regions
gcctccaccaagggcccatcggtcttccccctggcaccctcctccaagagcacctctgggggcacagcagccctgggctgcctggtcaaggactacttccccgaaccggtgacggtgtcgtggaactcaggcgccctgaccagcggcgtgcacaccttcccggctgtcctacagtcctcaggactctactccctcagcagcgtggtgaccgtgccctccagcagcttgggcacccagacctacatctgcaacgtgaatcacaagcccagcaacaccaaggtggacaagaaagttgagcccaaatcttgtgacaaaactcacacatgcccaccgtgcccagcacctgaactcctggggggaccgtcagtcttcctcttccccccaaaacccaaggacaccctcatgatctcccggacccctgaggtcacatgcgtggtggtggacgtgagccacgaagaccctgaggtcaagttcaactggtacgtggacggcgtggaggtgcataatgccaagacaaagccgcgggaggagcagtacaacagcacgtaccgtgtggtcagcgtcctcaccgtcctgcaccaggactggctgaatggcaaggagtacaagtgcaaggtctccaacaaagccctcccagcccccatcgagaaaaccatctccaaagccaaagggcagccccgagaaccacaggtgtacaccctgcccccatcccgggatgagctgaccaagaaccaggtcagcctgacctgcctggtcaaaggcttctatcccagcgacatcgccgtggagtgggagagcaatgggcagccggagaacaactacaagaccacgcctcccgtgctggactccgacggctccttcttcctctacagcaagctcaccgtggacaagagcaggtggcagcaggggaacgtcttctcatgctccgtgatgcatgaggctctgcacaaccactacacacagaagagcctctccctgtctccgggtaaa

SEQ ID NO: 56 - DNA, 321 bp, Artificial Sequence
  Light chain constant regions
cgtacggtggctgcaccatctgtcttcatcttcccgccatctgatgagcagttgaaatctggaactgcctctgttgtgtgcctgctgaataacttctatcccagagaggccaaagtacagtggaaggtggataacgccctccaatcgggtaactcccaggagagtgtcacagagcaggacagcaaggacagcacctacagcctcagcagcaccctgacgctgagcaaagcagactacgagaaacacaaagtctacgcctgcgaagtcacccatcagggcctgagttcgcccgtcacaaagagcttcaacaggggagagtgt

SEQ ID NO: 57 - DNA, 89 bp, Artificial Sequence
  ECL-2B7-S-H-5' primer
gacgaattcactctaaccatggaatggagctgggtctttctcttcttcctgtcagtaactacaggtgtccactccgagatcaccctgaa

SEQ ID NO: 58 - DNA, 93 bp, Artificial Sequence
  ECL-2B7-S-H-3' primer
ctcaggctgaagccgctgaaggtgcaggtcagggtcagggtctgggtgggcttcaccagggtggggccgctctccttcagggtgatctcggag

SEQ ID NO: 59 - DNA, 90 bp, Artificial Sequence
  ECL-2B7-HC-1-5' primer
cagcggcttcagcctgagcacttatggtataggagtaagctggatcaggcagccccccggcaaggccctggagtggctggcccacatttg

SEQ ID NO: 60 - DNA, 95 bp, Artificial Sequence
  ECL-2B7-HC-1-3' primer
cctggttcttgctggtgtccttggtgatggtcagcctgctcttcagggctgtgttatagtacttattatcattccaccaaatgtgggccagccac

SEQ ID NO: 61 - DNA, 90 bp, Artificial Sequence
  ECL-2B7-HC-2-5' primer
acaccagcaagaaccaggtggtgctgaccatgaccaacatggaccccgtggacaccgccacctactactgcgccaggaaggagggcagct

SEQ ID NO: 62 - DNA, 85 bp, Artificial Sequence
  ECL-2B7-HC-2-3' primer
gggcccttggtggaggcgctgctcacggtcaccagggtgccctggccccagtaagcaaagggggccgagctgccctccttcctgg

SEQ ID NO: 63 - DNA, 20 bp, Artificial Sequence
  Ch57.H.C-5' primer
gacgaattcactctaaccat

SEQ ID NO: 64 - DNA, 25 bp, Artificial Sequence
  ECL-2B7-WH-3' primer
ttgggcccttggtggaggcgctgct

SEQ ID NO: 65 - DNA, 22 bp, Artificial Sequence
  h2B7-H.C-W55Y-5` primer
tttggtataatgataataagta

SEQ ID NO: 66 - DNA, 22 bp, Artificial Sequence
  h2B7-H.C-W55Y-3` primer
tcattataccaaatgtgggcca

SEQ ID NO: 67 - DNA, 22 bp, Artificial Sequence
  h2B7-H.C-W55S-5` primer
tttggtcgaatgataataagta

SEQ ID NO: 68 - DNA, 22 bp, Artificial Sequence
  h2B7-H.C-W55S-3` primer
tcattcgaccaaatgtgggcca

SEQ ID NO: 69 - DNA, 27 bp, Artificial Sequence
  h2B7-H.C-SLIC-5` primer
gccagtgtgctggaattcactctaacc

SEQ ID NO: 70 - DNA, 24 bp, Artificial Sequence
  h2B7-H.C-SLIC-3 primer
aagaccgatgggcccttggtggag

SEQ ID NO: 71 - DNA, 20 bp, Artificial Sequence
  h2B7-L.C-N31V-5` primer
ttttagtaagtagcaatcaa

SEQ ID NO: 72 - DNA, 22 bp, Artificial Sequence
  h2B7-L.C-N31V-3` primer
ctacttactaaaaggctctgac

SEQ ID NO: 73 - DNA, 20 bp, Artificial Sequence
  h2B7-L.C-N31F-5` primer
ttttattcagtagcaatcaa

SEQ ID NO: 74 - DNA, 22 bp, Artificial Sequence
  h2B7-L.C-N31F-3` primer
ctactgaataaaaggctctgac

SEQ ID NO: 75 - DNA, 31 bp, Artificial Sequence
  h2B7-L.C-SLIC 5` primer
atagggagacccaagcttcggcacgagcaga

SEQ ID NO: 76 - DNA, 29 bp, Artificial Sequence
  h2B7-L.C-SLIC 3` primer
tggtgcagccaccgtacgcttgatctcca

SEQ ID NO: 77 - protein, 16 aa, Artificial Sequence
  Hz2B7-1.0~4.0 CDR2
HIXXXDNKYYNTALKS

SEQ ID NO: 78 - protein, 16 aa, Artificial Sequence
  Hz2B7-1.0~4.0 CDR2
HIWXNDNKYYNTALKS

SEQ ID NO: 79 - protein, 17 aa, Artificial Sequence
  Hz2B7-0.1~0.3 CDR1
KSSQSLLXSSNQKNYLA

SEQ ID NO: 80 - protein, 9 aa, Artificial Sequence
  Hz2B7-0.1~0.3 CDR3
QQHYRXPPT